European Patent Specification EP 3 511 407 B1, published May 17, 2023. Title: CHRISTENSENELLA INTESTINIHOMINIS AND APPLICATION THEREOF. Applicant: BGI SHENZHEN. Application EP16915429.1 based on PCT/CN2016/098247. The sequence listing filed with the application follows.

SEQUENCE LISTING (3 sequences)

SEQ ID NO: 1 - DNA, 1366 bp, Christensenella intestinihominis AF73-05CM02
ttgctctttgtgaagccctcgggtggaactgcgagtatacttagtggcggacgggtgagtaacgcgtgagcaatctgccctgcaatgggggacaacagttggaaacgactgctaataccgcatgagaccacgaaaccgcatggttttgaggtaaaaggatttattcgatgcaggatgagctcgcgtcccattagatagttggtgaggtaacggcccaccaagtcaacgatgggtagccgacctgagagggtgatcggccacactggaactgagacacggtccagactcctacgggaggcagcagtggggaatattgggcaatgggggaaaccctgacccagcaacgccgcgtgagggaagaaggtcttcggattgtaaacctttgtcctatgggacgaaacaaatgacggtaccataggaggaagctccggctaactacgtgccagcagccgcggtaatacgtagggagcaagcgttgtccggaattactgggcgtaaagggtgcgtaggtggctatgtaagtcagatgtgaaagaccggggcttaaccccggggttgcatttgaaactgtgtggcttgagtacaggagagggaagtggaattcctagtgtagcggtgaaatgcgtagatattaggaggaacaccagtggcgaaggcgactttctggactgtaactgacactgaagcacgaaagcgtggggagcaaacaggattagataccctggtagtccacgccgtaaacgatggatactaggtgtggggcccgatagggttccgtgccgaagctaacgcattaagtatcccgcctggggagtacgatcgcaaggttgaaactcaaaggaattgacgggggcccgcacaagcagcggagcatgtggtttaattcgaagcaacgcgaagaaccttaccaaggcttgacatcctctgacgactgtagagatacagtttcccttcggggcagagagacaggtggtgcatggttgtcgtcagctcgtgtcgtgagatgttgggttaagtcccgcaacgagcgcaacccttattgctagttgccagcgcgtaaaggcgggaactctagtgagactgccggggacaactcggaggaaggtggggacgacgtcaaatcatcatgccccttatgtcttgggctacacacgtgctacaatggccggtacaaagggcagcgaacccgtaaggggaagcgaatctcaaaaagccggtcccagttcggattgtgggctgcaacccgcccacatgaagtcggagttgctagtaatcgcgaatcagcatgtcgcggtgaatgcgttcccgggccttgtacacaccgcccgtcacaccacggaagttgggagcacccgaagccagtgga

SEQ ID NO: 2 - DNA, 20 bp, artificial sequence
agagtttgatcatggctcag

SEQ ID NO: 3 - DNA, 22 bp, artificial sequence
tagggttaccttgttacgactt